European Patent Specification EP 3 534 966 B1, published June 19, 2024. Title: SynP198, a promoter for the specific expression of genes in direction selective retinal ganglion cells. Applicant: Friedrich Miescher Institute for Biomedical Research. The sequence listing filed with the application follows.

SEQUENCE LISTING (2 sequences)

SEQ ID NO: 1 - DNA, 426 bp, Mus musculus
ggttcattgtaagccactgtagtcgtgggtgactcacatcaaaccaccccttcgggaacacgatgccgacactgaaactacataggggagagcaaataaaactgtcttctctagtttggggaaattggagcctgccttagggaaacagtgactaatttacagctagtgtttggaatgagatcatctgtcaaaataaatgtatctttacttccttcttgagaggaagcaagctgttttatgatgttccttggaatccttaaaaatacagagcaacatttacattattaatgatacgctttattgctgcaggctaactaggtccaaaattgtccttccatagatggagctggagagttacacagaagtttgcatatcgagctcttaggtctgcatgtacagctaatgtacttgtggaccctgtcacat

SEQ ID NO: 2 - DNA, 106 bp, Mus musculus
atcctcacatggtcctgctggagttagtagagggtatataatggaagctcgacttccagctatcacatccactgtgttgttgtgaactggaatccactataggcca